European Patent Specification EP 3 840 767 B1, published November 15, 2023. Title: Peptides. Applicant: Hubro Therapeutics AS. The sequence listing filed with the application follows.

SEQUENCE LISTING (32 sequences)

SEQ ID NO: 1 - protein, 567 aa, Homo sapiens
MGRGLLRGLWPLHIVLWTRIASTIPPHVQKSVNNDMIVTDNNGAVKFPQLCKFCDVRFSTCDNQKSCMSNCSITSICEKPQEVCVAVWRKNDENITLETVCHDPKLPYHDFILEDAASPKCIMKEKKKPGETFFMCSCSSDECNDNIIFSEEYNTSNPDLLLVIFQVTGISLLPPLGVAISVIIIFYCYRVNRQQKLSSTWETGKTRKLMEFSEHCAIILEDDRSDISSTCANNINHNTELLPIELDTLVGKGRFAEVYKAKLKQNTSEQFETVAVKIFPYEEYASWKTEKDIFSDINLKHENILQFLTAEERKTELGKQYWLITAFHAKGNLQEYLTRHVISWEDLRKLGSSLARGIAHLHSDHTPCGRPKMPIVHRDLKSSNILVKNDLTCCLCDFGLSLRLDPTLSVDDLANSGQVGTARYMAPEVLESRMNLENVESFKQTDVYSMALVLWEMTSRCNAVGEVKDYEPPFGSKVREHPCVESMKDNVLRDRGRPEIPSFWLNHQGIQMVCETLTECWDHDPEARLTAQCVAERFSELEHLDRLSGRSCSEEKIPEDGSLNTTK

SEQ ID NO: 2 - protein, 161 aa, Homo sapiens
MGRGLLRGLWPLHIVLWTRIASTIPPHVQKSVNNDMIVTDNNGAVKFPQLCKFCDVRFSTCDNQKSCMSNCSITSICEKPQEVCVAVWRKNDENITLETVCHDPKLPYHDFILEDAASPKCIMKEKKSLVRLSSCVPVALMSAMTTSSSQKNITPAILTCC

SEQ ID NO: 3 - protein, 33 aa, Homo sapiens
KCIMKEKKSLVRLSSCVPVALMSAMTTSSSQKN

SEQ ID NO: 4 - protein, 24 aa, Homo sapiens
KCIMKEKKSLVRLSSCVPVALMSA

SEQ ID NO: 5 - protein, 24 aa, Artificial Sequence
  Modified peptide
KGIMKEKKSLVRLSSCVPVALMSA

SEQ ID NO: 6 - protein, 20 aa, Homo sapiens
SSCVPVALMSAMTTSSSQKN

SEQ ID NO: 7 - protein, 20 aa, Artificial Sequence
  Modified peptide
SSGVPVALMSAMTTSSSQKN

SEQ ID NO: 8 - protein, 161 aa, Artificial Sequence
  Modified peptide
  VARIANT 121: Any amino acid except cysteine
  VARIANT 135: Any amino acid except cysteine
MGRGLLRGLWPLHIVLWTRIASTIPPHVQKSVNNDMIVTDNNGAVKFPQLCKFCDVRFSTCDNQKSCMSNCSITSICEKPQEVCVAVWRKNDENITLETVCHDPKLPYHDFILEDAASPKXIMKEKKSLVRLSSXVPVALMSAMTTSSSQKNITPAILTCC

SEQ ID NO: 9 - protein, 9 aa, Homo sapiens
RLSSCVPVA

SEQ ID NO: 10 - protein, 23 aa, Homo sapiens
SLVRLSSCVPVALMSAMTTSSSQ

SEQ ID NO: 11 - protein, 22 aa, Homo sapiens
SPKCIMKEKKSLVRLSSCVPVA

SEQ ID NO: 12 - protein, 19 aa, Homo sapiens
PKCIMKEKKKSLVRLSSCV

SEQ ID NO: 13 - protein, 9 aa, Homo sapiens
SLVRLSSCV

SEQ ID NO: 14 - protein, 23 aa, Homo sapiens
ALMSAMTTSSSQKNITPAILTCC

SEQ ID NO: 15 - protein, 19 aa, Homo sapiens
AMTTSSSQKNITPAILTCC

SEQ ID NO: 16 - protein, 33 aa, Homo sapiens
SPKCIMKEKKSLVRLSSCVPVALMSAMTTSSSQ

SEQ ID NO: 17 - protein, 15 aa, Homo sapiens
KKSLVRLSSCVPVAL

SEQ ID NO: 18 - protein, 15 aa, Homo sapiens
VALMSAMTTSSSQKN

SEQ ID NO: 19 - protein, 15 aa, Homo sapiens
PVALMSAMTTSSSQK

SEQ ID NO: 20 - protein, 15 aa, Homo sapiens
KCIMKEKKSLVRLSS

SEQ ID NO: 21 - protein, 15 aa, Homo sapiens
CVPVALMSAMTTSSS

SEQ ID NO: 22 - protein, 15 aa, Homo sapiens
LVRLSSCVPVALMSA

SEQ ID NO: 23 - protein, 15 aa, Homo sapiens
MKEKKSLVRLSSCVP

SEQ ID NO: 24 - protein, 15 aa, Homo sapiens
KSLVRLSSCVPVALM

SEQ ID NO: 25 - protein, 15 aa, Homo sapiens
SSCVPVALMSAMTTS

SEQ ID NO: 26 - protein, 17 aa, Homo sapiens
KCIMKEKKSLVRLSSCV

SEQ ID NO: 27 - protein, 14 aa, Homo sapiens
VRLSSCVPVALMSA

SEQ ID NO: 28 - protein, 17 aa, Artificial Sequence
  Modified peptide
KGIMKEKKSLVRLSSCV

SEQ ID NO: 29 - protein, 9 aa, Homo sapiens
LVRLSSCVP

SEQ ID NO: 30 - protein, 9 aa, Artificial Sequence
  Modified peptide
LVRLSSGVP

SEQ ID NO: 31 - protein, 25 aa, Homo sapiens
RNRIPAVLRTEGEPLHTPSVGMRET

SEQ ID NO: 32 - protein, 25 aa, Homo sapiens
KTILKKAGIGMCVKVSSIFFINKQK